European Patent Specification EP 3 495 817 B1, published October 16, 2024. Title: MOLECULAR DIAGNOSTIC SCREENING ASSAY. Applicant: Raindance Technologies. The sequence listing filed with the application follows.

SEQUENCE LISTING (7 sequences)

SEQ ID NO: 1 - DNA, 58 bp, Artificial Sequence
  Synthetic Sequence
gatcgacgagacactctcgcagacctgctggtgagaggccagcaccatgcaactcctt

SEQ ID NO: 2 - DNA, 46 bp, Artificial Sequence
  Synthetic Sequence
cagcaacagcagcaggaagcagtatcatcgccgggagatataccca

SEQ ID NO: 3 - DNA, 64 bp, Artificial Sequence
  Synthetic Sequence
gatcgacgagacactctcgcagacctgctggtgagattgtttcttcattctatagcccagttgg

SEQ ID NO: 4 - DNA, 47 bp, Artificial Sequence
  Synthetic Sequence
ggattactgcatgaccaccaatgacagatcgccgggagatataccca

SEQ ID NO: 5 - DNA, 19 bp, Artificial Sequence
  Synthetic Sequence
gatcgacgagacactctcg

SEQ ID NO: 6 - DNA, 20 bp, Artificial Sequence
  Synthetic Sequence
tgggtatatctcccggcgat

SEQ ID NO: 7 - DNA, 17 bp, Artificial Sequence
  Synthetic Sequence
  n (1)..(17): Wherein n is selected from A, G, T, C
  misc_feature (1)..(1): n is a, c, g, or t
  misc_feature (5)..(5): n is a, c, g, or t
  misc_feature (7)..(7): n is a, c, g, or t
  misc_feature (10)..(10): n is a, c, g, or t
  misc_feature (12)..(12): n is a, c, g, or t
  misc_feature (15)..(15): n is a, c, g, or t
ncctngnctngngtnga